European Patent Application EP 4 763 189 A1, published June 24, 2026. Title: Functionalized biocatalytical compositions comprising pancreatic enzymes. Applicant: Perseo Pharma AG. The sequence listing filed with the application follows.

SEQUENCE LISTING (1 sequence)

SEQ ID NO: 1 - protein, 31 aa, synthetic construct
ELGGRGGGGGGGGGREGGGEREGGGGNGGGG